European Patent Specification EP 4 041 913 B1, published November 29, 2023. Title: NOVEL METHOD. Applicant: Babraham Institute. The sequence listing filed with the application follows.

SEQUENCE LISTING (17 sequences)

SEQ ID NO: 1 - DNA, 19 bp, Artificial Sequence
  synthetic
  misc_feature (1)..(1): 5'-[phos]
ctgtctcttatacacatct

SEQ ID NO: 2 - DNA, 34 bp, Artificial Sequence
  synthetic
gtctcgtgggctcggagatgtgtataagagacag

SEQ ID NO: 3 - DNA, 33 bp, Artificial Sequence
  synthetic
tcgtcggcagcgtcagatgtgtataagagacag

SEQ ID NO: 4 - DNA, 47 bp, Artificial Sequence
  synthetic
caagcagaagacggcatacgagattaaggcgagtctcgtgggctcgg

SEQ ID NO: 5 - DNA, 47 bp, Artificial Sequence
  synthetic
caagcagaagacggcatacgagatcgtactaggtctcgtgggctcgg

SEQ ID NO: 6 - DNA, 47 bp, Artificial Sequence
  synthetic
caagcagaagacggcatacgagatggactcctgtctcgtgggctcgg

SEQ ID NO: 7 - DNA, 47 bp, Artificial Sequence
  synthetic
caagcagaagacggcatacgagattaggcatggtctcgtgggctcgg

SEQ ID NO: 8 - DNA, 51 bp, Artificial Sequence
  synthetic
aatgatacggcgaccaccgagatctacactatcctcttcgtcggcagcgtc

SEQ ID NO: 9 - DNA, 51 bp, Artificial Sequence
  synthetic
aatgatacggcgaccaccgagatctacacagagtagatcgtcggcagcgtc

SEQ ID NO: 10 - DNA, 30 bp, Artificial Sequence
  synthetic
  misc_feature (30)..(30): /3ddC/
tcgtcggcagcgtcagatgtgtataagaga

SEQ ID NO: 11 - DNA, 31 bp, Artificial Sequence
  synthetic
  misc_feature (31)..(31): /3ddC/
gtctcgtgggctcggagatgtgtataagaga

SEQ ID NO: 12 - DNA, 33 bp, Artificial Sequence
  synthetic
ctgtctcttatacacatctgacgctgccgacga

SEQ ID NO: 13 - DNA, 29 bp, Artificial Sequence
  synthetic
gtgtagatctcggtggtcgccgtatcatt

SEQ ID NO: 14 - DNA, 29 bp, Artificial Sequence
  synthetic
aatgatacggcgaccaccgagatctacac

SEQ ID NO: 15 - DNA, 34 bp, Artificial Sequence
  synthetic
ctgtctcttatacacatctccgagcccacgagac

SEQ ID NO: 16 - DNA, 24 bp, Artificial Sequence
  synthetic
caagcagaagacggcatacgagat

SEQ ID NO: 17 - DNA, 24 bp, Artificial Sequence
  synthetic
atctcgtatgccgtcttctgcttg